European Patent Application EP 4 400 578 A1, published July 17, 2024. Title: 乳酸菌、乳酸菌スターター、発酵乳、発酵乳の製造方法、及び乳酸菌のスクリーニング方法. Applicant: Meiji Co., Ltd. Application JP. The sequence listing filed with the application follows.

SEQUENCE LISTING (2 sequences)

SEQ ID NO: 1 - DNA, 20 bp, synthetic construct
  source 1..20: mol_type = other DNA; note = Fprimer
gacttgaagaaacagcgcgt

SEQ ID NO: 2 - DNA, 20 bp, synthetic construct
  source 1..20: mol_type = other DNA; note = Rprimer
taggtggaggcgttacagtg